European Patent Application EP 4 467 644 A1, published November 27, 2024. Title: アミダイトモノマー. Applicant: 国立大学法人東海国立大学機構. The sequence listing filed with the application follows.

SEQUENCE LISTING (1 sequence)

SEQ ID NO: 1 - DNA, 21 bp, synthetic construct
  misc_feature 1..21: note = SNA polynucleotide
  misc_feature 2: note = n is diaminopurine
  misc_feature 3: note = n is diaminopurine
  misc_feature 5: note = n is diaminopurine
  misc_feature 6: note = n is thiouracil
  misc_feature 8: note = n is diaminopurine
  misc_feature 12: note = n is thiouracil
  misc_feature 14: note = n is diaminopurine
  misc_feature 15: note = n is thiouracil
  misc_feature 16: note = n is diaminopurine
  misc_feature 17: note = n is diaminopurine
  source 1..21: mol_type = other DNA
cnncnncngtcngnnnngcta